European Patent Specification EP 3 871 222 B1, published January 1, 2025. Title: Vector-Based Haplotype Identification. Applicant: KWS SAAT SE & Co. KGaA. The sequence listing filed with the application follows.

SEQUENCE LISTING (35 sequences)

SEQ ID NO: 1 - DNA, 49 bp, Artificial Sequence
  50 nucleotide (nt) position wide sub-sequence of Genotype 1 (G1)
aataggtaatccctcggattggtgagcctctgatgttttaatattggat

SEQ ID NO: 2 - DNA, 50 bp, Artificial Sequence
  50 nucleotide (nt) position wide sub-sequence of Genotype 2 (G2)
aataggtaatcactcggattggttgagcctctgatgaattaataatggat

SEQ ID NO: 3 - DNA, 49 bp, Artificial Sequence; identical to SEQ ID NO: 1
  50 nucleotide (nt) position wide sub-sequence of Genotype 3 (G3)

SEQ ID NO: 4 - DNA, 50 bp, Artificial Sequence; identical to SEQ ID NO: 2
  50 nucleotide (nt) position wide sub-sequence of Genotype 4 (G4)

SEQ ID NO: 5 - DNA, 50 bp, Artificial Sequence; identical to SEQ ID NO: 2
  50 nucleotide (nt) position wide sub-sequence of Genotype 5 (G5)

SEQ ID NO: 6 - DNA, 50 bp, Artificial Sequence
  50 nucleotide (nt) position wide sub-sequence of Genotype 6 (G6)
aataggtaatctctcggattggttgagcctctgatgaattaatactggat

SEQ ID NO: 7 - DNA, 50 bp, Artificial Sequence; identical to SEQ ID NO: 2
  consensus of G1-G6

SEQ ID NO: 8 - DNA, 10 bp, Artificial Sequence
  sub-sequence of of a length of 10 nucleotide positions at the genomic location A1 derived from G1
aataggtaat

SEQ ID NO: 9 - DNA, 10 bp, Artificial Sequence
  sub-sequence of of a length of 10 nucleotide positions at the genomic location A1 derived from G2
aataggtaat

SEQ ID NO: 10 - DNA, 10 bp, Artificial Sequence
  sub-sequence of of a length of 10 nucleotide positions at the genomic location A1 derived from G3
aataggtaat

SEQ ID NO: 11 - DNA, 10 bp, Artificial Sequence
  sub-sequence of of a length of 10 nucleotide positions at the genomic location A1 derived from G4
aataggtaat

SEQ ID NO: 12 - DNA, 10 bp, Artificial Sequence
  sub-sequence of of a length of 10 nucleotide positions at the genomic location A1 derived from G5
aataggtaat

SEQ ID NO: 13 - DNA, 10 bp, Artificial Sequence
  sub-sequence of of a length of 10 nucleotide positions at the genomic location A1 derived from G6
aataggtaat

SEQ ID NO: 14 - DNA, 10 bp, Artificial Sequence
  sub-sequence of of a length of 10 nucleotide positions at the genomic location A2 derived from G1
ccctcggatt

SEQ ID NO: 15 - DNA, 10 bp, Artificial Sequence
  sub-sequence of of a length of 10 nucleotide positions at the genomic location A2 derived from G2
cactcggatt

SEQ ID NO: 16 - DNA, 10 bp, Artificial Sequence
  sub-sequence of of a length of 10 nucleotide positions at the genomic location A2 derived from G3
ccctcggatt

SEQ ID NO: 17 - DNA, 10 bp, Artificial Sequence
  sub-sequence of of a length of 10 nucleotide positions at the genomic location A2 derived from G4
cactcggatt

SEQ ID NO: 18 - DNA, 10 bp, Artificial Sequence
  sub-sequence of of a length of 10 nucleotide positions at the genomic location A2 derived from G5
cactcggatt

SEQ ID NO: 19 - DNA, 10 bp, Artificial Sequence
  sub-sequence of of a length of 10 nucleotide positions at the genomic location A2 derived from G6
ctctcggatt

SEQ ID NO: 20 - DNA, 10 bp, Artificial Sequence
  sub-sequence of of a length of 10 nucleotide positions at the genomic location A3 derived from G2
ggttgagcct

SEQ ID NO: 21 - DNA, 10 bp, Artificial Sequence
  sub-sequence of of a length of 10 nucleotide positions at the genomic location A3 derived from G4
ggttgagcct

SEQ ID NO: 22 - DNA, 10 bp, Artificial Sequence
  sub-sequence of of a length of 10 nucleotide positions at the genomic location A3 derived from G5
ggttgagcct

SEQ ID NO: 23 - DNA, 10 bp, Artificial Sequence
  sub-sequence of of a length of 10 nucleotide positions at the genomic location A3 derived from G6
ggttgagcct

SEQ ID NO: 24 - DNA, 10 bp, Artificial Sequence
  sub-sequence of of a length of 10 nucleotide positions at the genomic location A4 derived from G1
ctgatgtttt

SEQ ID NO: 25 - DNA, 10 bp, Artificial Sequence
  sub-sequence of of a length of 10 nucleotide positions at the genomic location A4 derived from G2
ctgatgaatt

SEQ ID NO: 26 - DNA, 10 bp, Artificial Sequence
  sub-sequence of of a length of 10 nucleotide positions at the genomic location A4 derived from G3
ctgatgtttt

SEQ ID NO: 27 - DNA, 10 bp, Artificial Sequence
  sub-sequence of of a length of 10 nucleotide positions at the genomic location A4 derived from G4
ctgatgaatt

SEQ ID NO: 28 - DNA, 10 bp, Artificial Sequence
  sub-sequence of of a length of 10 nucleotide positions at the genomic location A4 derived from G5
ctgatgaatt

SEQ ID NO: 29 - DNA, 10 bp, Artificial Sequence
  sub-sequence of of a length of 10 nucleotide positions at the genomic location A4 derived from G6
ctgatgaatt

SEQ ID NO: 30 - DNA, 10 bp, Artificial Sequence
  sub-sequence of of a length of 10 nucleotide positions at the genomic location A5 derived from G1
aatattggat

SEQ ID NO: 31 - DNA, 10 bp, Artificial Sequence
  sub-sequence of of a length of 10 nucleotide positions at the genomic location A5 derived from G2
aataatggat

SEQ ID NO: 32 - DNA, 10 bp, Artificial Sequence
  sub-sequence of of a length of 10 nucleotide positions at the genomic location A5 derived from G3
aatattggat

SEQ ID NO: 33 - DNA, 10 bp, Artificial Sequence
  sub-sequence of of a length of 10 nucleotide positions at the genomic location A5 derived from G4
aataatggat

SEQ ID NO: 34 - DNA, 10 bp, Artificial Sequence
  sub-sequence of of a length of 10 nucleotide positions at the genomic location A5 derived from G5
aataatggat

SEQ ID NO: 35 - DNA, 10 bp, Artificial Sequence
  sub-sequence of of a length of 10 nucleotide positions at the genomic location A5 derived from G6
aatactggat